European Patent Specification EP 3 258 774 B1, published April 8, 2026. Title: MODIFICATION OF TRANSCRIPTIONAL REPRESSOR BINDING SITE IN NF-YC4 PROMOTER FOR INCREASED PROTEIN CONTENT AND RESISTANCE TO STRESS. Applicant: IOWA STATE UNIVERSITY RESEARCH FOUNDATION, INC. The sequence listing filed with the application follows.

SEQUENCE LISTING (20 sequences)

SEQ ID NO: 1 - DNA, 1447 bp, Oryza sativa
gcaagaaccccagttgagagtggagatggccattttgttcaggcactaggcagtgggtaggacggtgaggagtgtgtcctgcactcctgcttcccctgacgatcgatccccatgcgtgccgaagcatctgatacttttgctgtgctgttctttaatttaccctgatacttttggatatctgaagcagtagagctcgttcactcaaacaggctagcctgttttgctttctggtaagaacttaattaactagttgagatcgacatgcatggatgcgtgaatctattgttgcattttttctaatggatagttagatttgttccagctttttttttgtcaattctgttacatttgcagtgtcttcaacttctgcatcattcttctctattcttccttcactttctttcttgaactagaaaagcaaaccagagttctttttccccctcttctacataaacgaaaacagcttgttgactggctccctagagctttttgtaagttgatcatcgaagtagctagttctcttcacttatcagtcatcactgttctatgttctatctgcattttccttgattttgtacttttcctgaacgaaaggacaatccttagccatcataatgctatgatcgacttattctgaagtcatccggcctcgatcctcttttgtttcggtgagatctgtaatggtttaggaaaattatggatctctgaaaaataagaaacatctagtagtatatgaaattaagaaatgtcggaccacgtcaaatcctactggtatcatataccagataactaactttttgaatggaaccaaacacgagattgtgaatatatagcagtaagaaatacaaccccgaagggtaaaggagaaaaaggaaaagcagtttagtgtacgagctgtaggagtagctttgctcctgccaaggcccagatccttgcctcttccttcatttctgcgaggagaccaggcactgaggtctcattgtgatcgaagattctcctgtttctctccttccagatctcctttgggaacaccctgtgtgtttgcaagcgcttagcttcattttcatgcatgatatgatctctggatagaagataagtagcccccacacatgcacttcgccacctatagccagcctcgagttctcatctgtttgatccgtcgcacatgtggagcaacgaagctctagagtacgtctcctaatctctacttacttttgcagtttgcacacatattgagaaatgcttatcaatccttcgatctctcacagacaatacctacaagcgtcgtttacactttgcatgtatagctagccattgttacatacgtggagcatgtagcgatcattcgttcctagcacgtaaattaatcgccgtaattttgcccatgcagacacagcacacacagctacaaatcgactgtaattaaggtacgtatatataggtgaca

SEQ ID NO: 2 - DNA, 1441 bp, Oryza sativa
gcaagaaccccagttgagagtggagatggccattttgttcaggcactaggcagtgggtaggacggtgaggagtgtgtcctgcactcctgcttcccctgacgatcgatccccatgcgtgccgaagcatctgatacttttgctgtgctgttctttaatttaccctgatacttttggatatctgaagcagtagagctcgttcactcaaacaggctagcctgttttgctttctggtaagaacttaattaactagttgagatcgacatgcatggatgcgtgaatctatattttttctaatggatagttagatttgttccagctttttttttgtcaattctgttacatttgcagtgtcttcaacttctgcatcattcttctctattcttccttcactttctttcttgaactagaaaagcaaaccagagttctttttccccctcttctacataaacgaaaacagcttgttgactggctccctagagctttttgtaagttgatcatcgaagtagctagttctcttcacttatcagtcatcactgttctatgttctatctgcattttccttgattttgtacttttcctgaacgaaaggacaatccttagccatcataatgctatgatcgacttattctgaagtcatccggcctcgatcctcttttgtttcggtgagatctgtaatggtttaggaaaattatggatctctgaaaaataagaaacatctagtagtatatgaaattaagaaatgtcggaccacgtcaaatcctactggtatcatataccagataactaactttttgaatggaaccaaacacgagattgtgaatatatagcagtaagaaatacaaccccgaagggtaaaggagaaaaaggaaaagcagtttagtgtacgagctgtaggagtagctttgctcctgccaaggcccagatccttgcctcttccttcatttctgcgaggagaccaggcactgaggtctcattgtgatcgaagattctcctgtttctctccttccagatctcctttgggaacaccctgtgtgtttgcaagcgcttagcttcattttcatgcatgatatgatctctggatagaagataagtagcccccacacatgcacttcgccacctatagccagcctcgagttctcatctgtttgatccgtcgcacatgtggagcaacgaagctctagagtacgtctcctaatctctacttacttttgcagtttgcacacatattgagaaatgcttatcaatccttcgatctctcacagacaatacctacaagcgtcgtttacactttgcatgtatagctagccattgttacatacgtggagcatgtagcgatcattcgttcctagcacgtaaattaatcgccgtaattttgcccatgcagacacagcacacacagctacaaatcgactgtaattaaggtacgtatatataggtgaca

SEQ ID NO: 3 - DNA, 1439 bp, Oryza sativa
gcaagaaccccagttgagagtggagatggccattttgttcaggcactaggcagtgggtaggacggtgaggagtgtgtcctgcactcctgcttcccctgacgatcgatccccatgcgtgccgaagcatctgatacttttgctgtgctgttctttaatttaccctgatacttttggatatctgaagcagtagagctcgttcactcaaacaggctagcctgttttgctttctggtaagaacttaattaactagttgagatcgacatgcatggatgcgtgaatctattgttgcattttttctaatggatagttagatttgttccagctttttttttgtcaattctgttacatttgcagtgtcttcaacttctgcatcattcttctctattcttccttcactttctttcttgaactagaaaagcaaaccagagttctttttccccctcttctacataaacgaaaacagctggctccctagagctttttgtaagttgatcatcgaagtagctagttctcttcacttatcagtcatcactgttctatgttctatctgcattttccttgattttgtacttttcctgaacgaaaggacaatccttagccatcataatgctatgatcgacttattctgaagtcatccggcctcgatcctcttttgtttcggtgagatctgtaatggtttaggaaaattatggatctctgaaaaataagaaacatctagtagtatatgaaattaagaaatgtcggaccacgtcaaatcctactggtatcatataccagataactaactttttgaatggaaccaaacacgagattgtgaatatatagcagtaagaaatacaaccccgaagggtaaaggagaaaaaggaaaagcagtttagtgtacgagctgtaggagtagctttgctcctgccaaggcccagatccttgcctcttccttcatttctgcgaggagaccaggcactgaggtctcattgtgatcgaagattctcctgtttctctccttccagatctcctttgggaacaccctgtgtgtttgcaagcgcttagcttcattttcatgcatgatatgatctctggatagaagataagtagcccccacacatgcacttcgccacctatagccagcctcgagttctcatctgtttgatccgtcgcacatgtggagcaacgaagctctagagtacgtctcctaatctctacttacttttgcagtttgcacacatattgagaaatgcttatcaatccttcgatctctcacagacaatacctacaagcgtcgtttacactttgcatgtatagctagccattgttacatacgtggagcatgtagcgatcattcgttcctagcacgtaaattaatcgccgtaattttgcccatgcagacacagcacacacagctacaaatcgactgtaattaaggtacgtatatataggtgaca

SEQ ID NO: 4 - DNA, 1336 bp, Oryza sativa
gcaagaaccccagttgagagtggagatggccattttgttcaggcactaggcagtgggtaggacggtgaggagtgtgtcctgcactcctgcttcccctgacgatcgatccccatgcgtgccgaagcatctgatacttttgctgtgctgttctttaatttaccctgatacttttggatatctgaagcagtagagctcgttcactcaaacaggctagcctgttttgctttctggtaagaacttaattaactagttgagatcgacatgcatggatgcgtgaatctattgttgcattttttctaatggatagttagatttgttccagctttttttttgtcaattctgttacatttgcagtgtcttcaacttctgcatcattcttctctattcttccttcactttctttcttgaactagaaaagcaaaccagagttctttttccccctcttctacataaacgaaaacagcttgttgactggctccctagagctttttgtaagttgatcatcgaagtagctagttctcttcacttatctccggcctcgatcctcttttgtttcggtgagatctgtaatggtttaggaaaattatggatctctgaaaaataagaaacatctagtagtatatgaaattaagaaatgtcggaccacgtcaaatcctactggtatcatataccagataactaactttttgaatggaaccaaacacgagattgtgaatatatagcagtaagaaatacaaccccgaagggtaaaggagaaaaaggaaaagcagtttagtgtacgagctgtaggagtagctttgctcctgccaaggcccagatccttgcctcttccttcatttctgcgaggagaccaggcactgaggtctcattgtgatcgaagattctcctgtttctctccttccagatctcctttgggaacaccctgtgtgtttgcaagcgcttagcttcattttcatgcatgatatgatctctggatagaagataagtagcccccacacatgcacttcgccacctatagccagcctcgagttctcatctgtttgatccgtcgcacatgtggagcaacgaagctctagagtacgtctcctaatctctacttacttttgcagtttgcacacatattgagaaatgcttatcaatccttcgatctctcacagacaatacctacaagcgtcgtttacactttgcatgtatagctagccattgttacatacgtggagcatgtagcgatcattcgttcctagcacgtaaattaatcgccgtaattttgcccatgcagacacagcacacacagctacaaatcgactgtaattaaggtacgtatatataggtgaca

SEQ ID NO: 5 - DNA, 111 bp, Oryza sativa
agtcatcactgttctatgttctatctgcattttccttgattttgtacttttcctgaacgaaaggacaatccttagccatcataatgctatgatcgacttattctgaagtca

SEQ ID NO: 6 - DNA, 1257 bp, Oryza sativa
gcaagaaccccagttgagagtggagatggccattttgttcaggcactaggcagtgggtaggacggtgaggagtgtgtcctgcactcctgcttcccctgacgatcgatccccatgcgtgccgaagcatctgatacttttgctgtgctgttctttaatttaccctgatacttttggatatctgaagcagtagagctcgttcactcaaacaggctagcctgttttgctttctggtaagaacttaattaactagttgagatcgacatgcatggatgcgtgaatctattgttgcattttttctaatggatagttagatttgttccagctttttttttgtcaattctgttacatttgcagtgtcttcaacttctgcatcattcttctctattcttccttcactttctttcttgaactagaaaagcaaaccagagttctttttccccctcttctacatatccggcctcgatcctcttttgtttcggtgagatctgtaatggtttaggaaaattatggatctctgaaaaataagaaacatctagtagtatatgaaattaagaaatgtcggaccacgtcaaatcctactggtatcatataccagataactaactttttgaatggaaccaaacacgagattgtgaatatatagcagtaagaaatacaaccccgaagggtaaaggagaaaaaggaaaagcagtttagtgtacgagctgtaggagtagctttgctcctgccaaggcccagatccttgcctcttccttcatttctgcgaggagaccaggcactgaggtctcattgtgatcgaagattctcctgtttctctccttccagatctcctttgggaacaccctgtgtgtttgcaagcgcttagcttcattttcatgcatgatatgatctctggatagaagataagtagcccccacacatgcacttcgccacctatagccagcctcgagttctcatctgtttgatccgtcgcacatgtggagcaacgaagctctagagtacgtctcctaatctctacttacttttgcagtttgcacacatattgagaaatgcttatcaatccttcgatctctcacagacaatacctacaagcgtcgtttacactttgcatgtatagctagccattgttacatacgtggagcatgtagcgatcattcgttcctagcacgtaaattaatcgccgtaattttgcccatgcagacacagcacacacagctacaaatcgactgtaattaaggtacgtatatataggtgaca

SEQ ID NO: 7 - DNA, 190 bp, Oryza sativa
aacgaaaacagcttgttgactggctccctagagctttttgtaagttgatcatcgaagtagctagttctcttcacttatcagtcatcactgttctatgttctatctgcattttccttgattttgtacttttcctgaacgaaaggacaatccttagccatcataatgctatgatcgacttattctgaagtca

SEQ ID NO: 8 - DNA, 1176 bp, Glycine max
taatataatataagaatttgtaaattataaacctaaaaaaggtgcataccaaatgaatagtttatttcaaaagcaaagataaattttatacacaaaagtgacaaaatgtggacttgaaaatcacatgctagagcaaagcaaggttcagatgaagccaaatggctagaacgtaaatgctgcaaaaatcaattatatttgaatctcacgggcattgaacaaaagagaatggacccatcaatggggcattgacatggatggatggaacaccctcatagtcacatgccacaacagagtaacgctaaacaaaatgtattaacaaaaactataggatcatgctttcttaatttaaaaacataggtggtcagtttttgttaacattaatttttaggattatttgttgaagacaaatatggaaggtttataataatttatgtgcattactcaatgtaatccttaaaatgaaaataactaaactttttttttttggatagttaaacaactacgaagctaaatgaataattaaatcaatattaattttgattaaaaataagattaataatatccctaatattgtgaacaaactttgttggtaatgtaaaaaaaattaaaagaaacaagattaaattacgtatttaataatttaagattaatgttgtttaatttgattttttaaatatttatctttcttttgaatttgattctttagttcacttaagattatgatcgttaataattctaaaagataaatgtcatcaatcttgaattgattgaaagattaaattaaataaaaagaattaagataaatgatgaaaatacatttaaaaaataagatgaaacaaaatgtgtcatttaaccaaaaaaaaaaggaaaaataaattaaaaaaaggaacttacccttcccctcaaaaaagaaaagaaaaaaaaaaaggaacttacccttggttgttccgttgaaattgaaaaaacaaaccctaaacttaccttaacctaggtcctagggcactggtcggatatgttattgtttagtttaccttatcccaccacatacatagttttttttttcttaaatttcccaatcaattccatccatcgggtctttactctcttacccaacccacacacactctttctctctctctctttccctgatcatcaaaatcagaaaaaattggggga

SEQ ID NO: 9 - DNA, 1159 bp, Glycine max
taatataatataagaatttgtaaattataaacctaaaaaaggtgcataccaaatgaatagtttatttcaaaagcaaagataaattttatacacaaaagtgacaaaatgtggacttgaaaatcacatgctagagcaaagcaaggttcagatgaagccaaatggctagaacgtaaatgctgcaaaaatcaattatatttgaatctcacgggcattgaacaaaagagaatggacccatcaatggggcattgacatggatggatggaacaccctcatgagtaacgctaaacaaaatgtattaacaaaaactataggatcatgctttcttaatttaaaaacataggtggtcagtttttgttaacattaatttttaggattatttgttgaagacaaatatggaaggtttataataatttatgtgcattactcaatgtaatccttaaaatgaaaataactaaactttttttttttggatagttaaacaactacgaagctaaatgaataattaaatcaatattaattttgattaaaaataagattaataatatccctaatattgtgaacaaactttgttggtaatgtaaaaaaaattaaaagaaacaagattaaattacgtatttaataatttaagattaatgttgtttaatttgattttttaaatatttatctttcttttgaatttgattctttagttcacttaagattatgatcgttaataattctaaaagataaatgtcatcaatcttgaattgattgaaagattaaattaaataaaaagaattaagataaatgatgaaaatacatttaaaaaataagatgaaacaaaatgtgtcatttaaccaaaaaaaaaaggaaaaataaattaaaaaaaggaacttacccttcccctcaaaaaagaaaagaaaaaaaaaaaggaacttacccttggttgttccgttgaaattgaaaaaacaaaccctaaacttaccttaacctaggtcctagggcactggtcggatatgttattgtttagtttaccttatcccaccacatacatagttttttttttcttaaatttcccaatcaattccatccatcgggtctttactctcttacccaacccacacacactctttctctctctctctttccctgatcatcaaaatcagaaaaaattggggga

SEQ ID NO: 10 - DNA, 17 bp, Glycine max
agtcacatgccacaaca

SEQ ID NO: 11 - DNA, 1135 bp, Glycine max
taatataatataagaatttgtaaattataaacctaaaaaaggtgcataccaaatgaatagtttatttcaaaagcaaagataaattttatacacaaaagtgacaaaatgtggacttgaaaatcacatgctagagcaaagcaaggttcagatgaagccaaatggctagaacgtaaatgctgcaaaaatcaattatatttgaatctcacgggcattgaacaaaagagaatggacccatcaatggggcattgacatggatggatggaacaccctcatagtcacatgccacaacagagtaacgctaaacaaaatgtattaacaaaaactataggatcatgctttcttaatttaaaaacataggtaagacaaatatggaaggtttataataatttatgtgcattactcaatgtaatccttaaaatgaaaataactaaactttttttttttggatagttaaacaactacgaagctaaatgaataattaaatcaatattaattttgattaaaaataagattaataatatccctaatattgtgaacaaactttgttggtaatgtaaaaaaaattaaaagaaacaagattaaattacgtatttaataatttaagattaatgttgtttaatttgattttttaaatatttatctttcttttgaatttgattctttagttcacttaagattatgatcgttaataattctaaaagataaatgtcatcaatcttgaattgattgaaagattaaattaaataaaaagaattaagataaatgatgaaaatacatttaaaaaataagatgaaacaaaatgtgtcatttaaccaaaaaaaaaaggaaaaataaattaaaaaaaggaacttacccttcccctcaaaaaagaaaagaaaaaaaaaaaggaacttacccttggttgttccgttgaaattgaaaaaacaaaccctaaacttaccttaacctaggtcctagggcactggtcggatatgttattgtttagtttaccttatcccaccacatacatagttttttttttcttaaatttcccaatcaattccatccatcgggtctttactctcttacccaacccacacacactctttctctctctctctttccctgatcatcaaaatcagaaaaaattggggga

SEQ ID NO: 12 - DNA, 41 bp, Glycine max
ggtcagtttttgttaacattaatttttaggattatttgttg

SEQ ID NO: 13 - DNA, 1105 bp, Glycine Max
taatataatataagaatttgtaaattataaacctaaaaaaggtgcataccaaatgaatagtttatttcaaaagcaaagataaattttatacacaaaagtgacaaaatgtggacttgaaaatcacatgctagagcaaagcaaggttcagatgaagccaaatggctagaacgtaaatgctgcaaaaatcaattatatttgaatctcacgggcattgaacaaaagagaatggacccatcaatggggcattgacatggatggatggaacaccctcatagtcacatgccacaacagagtaacgctaaacaaaatgtattaacaaaaactataggatcatgctttcttaatttaaaaacataggtggtcagtttttgttaacattaatttttaggattatttgttgaagacaaatatggaaggtttataataatttatgtgcattactcaatgtaatccttaaaatgaaaataactaaactttttttttttggatagttaaacaactacgaagctaaatgaataattaaatcaatattaattttgattaaaaataagattaataatatccctaatattgtgaacaaactttttaatttgattttttaaatatttatctttcttttgaatttgattctttagttcacttaagattatgatcgttaataattctaaaagataaatgtcatcaatcttgaattgattgaaagattaaattaaataaaaagaattaagataaatgatgaaaatacatttaaaaaataagatgaaacaaaatgtgtcatttaaccaaaaaaaaaaggaaaaataaattaaaaaaaggaacttacccttcccctcaaaaaagaaaagaaaaaaaaaaaggaacttacccttggttgttccgttgaaattgaaaaaacaaaccctaaacttaccttaacctaggtcctagggcactggtcggatatgttattgtttagtttaccttatcccaccacatacatagttttttttttcttaaatttcccaatcaattccatccatcgggtctttactctcttacccaacccacacacactctttctctctctctctttccctgatcatcaaaatcagaaaaaattggggga

SEQ ID NO: 14 - DNA, 71 bp, Glycine max
tgttggtaatgtaaaaaaaattaaaagaaacaagattaaattacgtatttaataatttaagattaatgttg

SEQ ID NO: 15 - DNA, 586 bp, Arabidopsis thaliana
ctcagaagaagcctcctttcgatctgtcagccattgaagaaacctcctttcgatctgtcagccattgaagatcagaagaaacaagactcacacggtcagccattgaagaagcctcctctcattacctctcatcaaacatctagatctgtacccaaaccttatccctttttccttatttctcgctttgtctattcttaatctgattaatacttgttgttgttccaggttatagaagatctgggttgtgttatatgcttcattttctccacagcgaccagttggtgtttggttcttagattcatgaagaccaatagagagcaggaaatttacgttgaaagaagcttcaaaccaaacaattcaacaattcagaatttgatggacattgaaaggttcattttgcctcacacttctacatcaggtgtcgcaaggctcaaaatgagggtcatatcatgggtcgggcttcagttctacaactactgatattgggccttatcacaaattagttatagggccattgtatccaatatttaatatctctgtaaacttgtttaatggttattttgttctaatgcccattacaactaga

SEQ ID NO: 16 - protein, 59 aa, Arabidopsis thaliana
MKTNREQEIYVERSFKPNNSTIQNLMDIERFILPHTSTSGVARLKMRVISWVGLQFYNY

SEQ ID NO: 17 - DNA, 32 bp, Glycine max
ggtcagtttttgttaacattaatttttaggat

SEQ ID NO: 18 - DNA, 20 bp, Artificial
  Synthetic
cctcccaggcatggcagtcc

SEQ ID NO: 19 - DNA, 18 bp, Artificial
  Synthetic
ccatcaaggctccgctgg

SEQ ID NO: 20 - DNA, 1034 bp, Zea mays
agggccctgcagcggcggcagctggcgggagagaggcttgggactgggccgcccggccgcgaggaataaactcactcctgtcttcatacgtatccatagccggcaggcggcagtacctgtatgtggttttagctatacgcgacctcagttcgggcgcaaggttagtcttcgatttaagcatagattttattttatcttcttggctccaccaaataacactaacaaaatcgctttggcttctatgggttcaaattaagcactggatcgtaccattttcttgttcatttatactttgtcatccaatccacaccgattaatttctcacggtcaacaacgcatgaagttttcatttctgggaagaagcatgtattttttttatctccgactcgatctagtggtgagaggaggaagatgaatagtgcatgcatatgatatctagagaggcaccagatctagtggctccatgttctgttcgcgggctaagaaaaaacataaacaagcaggcgcctgaaaaatagctagtccctaactttttagaccaatctgtatgtttattttgacgatattggtatgaaaaagtctctcaagaacaatatacatatgcagcatgcatgtgcatggtataattataaattattagcagagtttagataagtaggcccccacgtctgcgctccgccacctacagcgagcctccctttcctccctccctgattcgtttgcacttgctgagagctcaacagaatttggtcaccgatttcaattcgcagctactaattctcaccacattgaaattttcgatttgaaacagtacaatttctgaagagaaattgtacgtctgaaacggttgcatgtgtactatgaactgctagccattccctgcatacgtgggacacgctcagatcattcattcgcagcacgtacgtaaccttaatattctactatacatccatgcagctacaaccccgaccaggcgagaagaagcatcgatagtgtgacgagctaacccaccaccagcaacgtaatccaaatcc